European Patent Application EP 4 219 564 A1, published August 2, 2023. Title: WNT SIGNALING AGONIST MOLECULES. Applicant: THE BOARD OF TRUSTEES OF THE LELAND STANFORD JUNIOR UNIVERSITY. Application EP, filed September 11, 2015. The sequence listing filed with the application follows.

SEQUENCE LISTING (39 sequences)

SEQ ID NO: 1 - protein, 10 aa, synthetic construct
  REGION 1..10: note = synthetic amino acid sequence
GFTFSHYTLS

SEQ ID NO: 2 - protein, 17 aa, synthetic construct
  REGION 1..17: note = synthetic amino acid sequence
VISGDGSYTYYADSVKG

SEQ ID NO: 3 - protein, 9 aa, synthetic construct
  REGION 1..9: note = synthetic amino acid sequence
NFIKYVFAN

SEQ ID NO: 4 - protein, 11 aa, synthetic construct
  REGION 1..11: note = synthetic amino acid sequence
SGDKLGKKYAS

SEQ ID NO: 5 - protein, 8 aa, synthetic construct
  REGION 1..8: note = synthetic amino acid sequence
EKDNRPSG

SEQ ID NO: 6 - protein, 9 aa, synthetic construct
  REGION 1..9: note = synthetic amino acid sequence
SSFAGNSLE

SEQ ID NO: 7 - protein, 11 aa, synthetic construct
  REGION 1..11: note = synthetic amino acid sequence
SGDNIGSFYVH

SEQ ID NO: 8 - protein, 8 aa, synthetic construct
  REGION 1..8: note = synthetic amino acid sequence
DKSNRPSG

SEQ ID NO: 9 - protein, 9 aa, synthetic construct
  REGION 1..9: note = synthetic amino acid sequence
QSYANTLSL

SEQ ID NO: 10 - protein, 381 aa, synthetic construct
  REGION 1..381: note = synthetic amino acid sequence
MLLVNQSHQGFNKEHTSKMVSAIVLYVLLAAAAHSAFAADPIELTQPPSVSVAPGQTARISCSGDNIGSFYVHWYQQKPGQAPVLVIYDKSNRPSGIPERFSGSNSGNTATLTISGTQAEDEADYYCQSYANTLSLVFGGGTKLTVLGTTAASGSSGGSSSGAEVQLVESGGGLVQPGGSLRLSCAASGFTFSHYTLSWVRQAPGKGLEWVSVISGDGSYTYYADSVKGRFTISSDNSKNTLYLQMNSLRAEDTAVYYCARNFIKYVFANWGQGTLVTVSGSGSGKMYHTKGQEGSVCLRSSDCASGLCCARHFWSKICKPVLKEGQVCTKHRRKGSHGLEIFQRCYCGEGLSCRIQKDHHQASNSSRLHTCQRHHHHHHH

SEQ ID NO: 11 - protein, 6 aa, synthetic construct
  REGION 1..6: note = synthetic amino acid sequence
LLERIY

SEQ ID NO: 12 - protein, 6 aa, synthetic construct
  REGION 1..6: note = synthetic amino acid sequence
TLERVY

SEQ ID NO: 13 - protein, 6 aa, synthetic construct
  REGION 1..6: note = synthetic amino acid sequence
LLINIY

SEQ ID NO: 14 - protein, 15 aa, synthetic construct
  REGION 1..15: note = synthetic amino acid sequence
KYAAAVAAFAAAAGF

SEQ ID NO: 15 - protein, 15 aa, synthetic construct
  REGION 1..15: note = synthetic amino acid sequence
KYVAAVATFALQAGF

SEQ ID NO: 16 - protein, 15 aa, synthetic construct
  REGION 1..15: note = synthetic amino acid sequence
KYKELVKEFVGDAVE

SEQ ID NO: 17 - protein, 123 aa, synthetic construct
  REGION 1..123: note = synthetic amino acid sequence
MGVSFSEVMGKQKDEQAREQLKEGMKKIEEQGKKLSETRTQEELQKYAAAVAAFAAAAGFLGKNLEERRGFNRRGKEEIGKISGEVYKKLLDLKKAVRAKEKKGLDILNMVGEIKGLLERIYA

SEQ ID NO: 18 - protein, 123 aa, synthetic construct
  REGION 1..123: note = synthetic amino acid sequence
MGVSFSEVMGKQKDEQAREQLKEGMIKIEEQGKKLSETRTQEELQKYVAAVATFALQAGFLGPNLEERRGFNRRGKEEIGKISGEVYLKLLDLKKAVRAKEKKGLDILNMVGEIKGTLERVYA

SEQ ID NO: 19 - protein, 6 aa, synthetic construct
  REGION 1..6: note = synthetic amino acid sequence
GSGSGS

SEQ ID NO: 20 - protein, 5 aa, synthetic construct
  REGION 1..5: note = synthetic amino acid sequence
GSGSG

SEQ ID NO: 21 - protein, 10 aa, synthetic construct
  REGION 1..10: note = synthetic amino acid sequence
GSGSGGSGSG

SEQ ID NO: 22 - protein, 15 aa, synthetic construct
  REGION 1..15: note = synthetic amino acid sequence
GSGSGGSGSGGSGSG

SEQ ID NO: 23 - protein, 7 aa, synthetic construct
  REGION 1..7: note = synthetic amino acid sequence
  SITE 6: note = misc_feature - Xaa can be any naturally occurring amino acid
PPPSPXS

SEQ ID NO: 24 - protein, 5 aa, synthetic construct
  REGION 1..5: note = synthetic amino acid sequence
PPPSP

SEQ ID NO: 25 - protein, 90 aa, Homo sapiens
KMYHTKGQEGSVCLRSSDCASGLCCARHFWSKICKPVLKEGQVCTKHRRKGSHGLEIFQRCYCGEGLSCRIQKDHHQASNSSRLHTCQRH

SEQ ID NO: 26 - protein, 88 aa, Homo sapiens
KMSHIKGHEGDPCLRSSDCIEGFCCARHFWTKICKPVLHQGEVCTKQRKKGSHGLEIFQRCDCAKGLSCKVWKDATYSSKARLHVCQK

SEQ ID NO: 27 - protein, 5 aa, synthetic construct
  REGION 1..5: note = synthetic amino acid sequence
GGGGS

SEQ ID NO: 28 - protein, 9 aa, synthetic construct
  REGION 1..9: note = synthetic amino acid sequence
GGGGGGGGG

SEQ ID NO: 29 - protein, 9 aa, synthetic construct
  REGION 1..9: note = synthetic amino acid sequence
EEEEEEEEE

SEQ ID NO: 30 - protein, 9 aa, synthetic construct
  REGION 1..9: note = synthetic amino acid sequence
SSSSSSSSS

SEQ ID NO: 31 - protein, 9 aa, synthetic construct
  REGION 1..9: note = synthetic amino acid sequence
GGGGGCPPC

SEQ ID NO: 32 - protein, 15 aa, synthetic construct
  REGION 1..15: note = synthetic amino acid sequence
GGGGSGGGGSGGGGS

SEQ ID NO: 33 - protein, 13 aa, synthetic construct
  REGION 1..13: note = synthetic amino acid sequence
SCVPLMRCGGCCN

SEQ ID NO: 34 - protein, 14 aa, synthetic construct
  REGION 1..14: note = synthetic amino acid sequence
PSCVPLMRCGGCCN

SEQ ID NO: 35 - protein, 9 aa, synthetic construct
  REGION 1..9: note = synthetic amino acid sequence
GDLIYRNQK

SEQ ID NO: 36 - protein, 23 aa, synthetic construct
  REGION 1..23: note = synthetic amino acid sequence
GGGGGGGGGPSCVPLMRCGGCCN

SEQ ID NO: 37 - protein, 14 aa, synthetic construct
  REGION 1..14: note = synthetic amino acid sequence
GSTSGSGKSSEGKG

SEQ ID NO: 38 - protein, 5 aa, synthetic construct
  REGION 1..5: note = synthetic amino acid sequence
  REGION >5: note = MISC_FEATURE - the sequence (1)..(5) may be repeated n times where n is an interger selected from 1, 2, 3, 4, 5, etc.
GGGGS

SEQ ID NO: 39 - protein, 145 aa, Bacillus halodurans
MDVQRVGKAGLHRVDSKKQQTAAGVSFSEVMGKQRDEKAYERLQALMSKIDDQGKLLSETRTIEELRKYKELVKEFVGDAVELGLRLEERRGFNRRGRTKIYKIVKEVDRKLLDLTDAVLAKEKKGLDILNMVGEIKGLLINIYA